European Patent Specification EP 3 525 828 B1, published December 25, 2024. Title: ANTI-EDB ANTIBODIES AND ANTIBODY-DRUG CONJUGATES. Applicant: Pfizer Inc. Hooper, Andrea Therese Marquette, Kimberly Ann Subramanyam, Chakrapani Gerber, Hans-Peter May, Chad Michael. The sequence listing filed with the application follows.

SEQUENCE LISTING (57 sequences)

SEQ ID NO: 1 - protein, 116 aa, Artificial Sequence [sequence omitted]

SEQ ID NO: 2 - DNA, 348 bp, Artificial Sequence
  Synthetic nucleotide sequence
gaggtgcagctgttggagtctgggggaggcttggtacagcctggggggtccctgagactctcctgtgcagcctctggattcacctttagcagtttttcgatgagctgggtccgccaggctccagggaaggggctggagtgggtctcatctattagtggtagttcgggtaccacatactacgcagactccgtgaagggccggttcaccatctccagagacaattccaagaacacgctgtatctgcaaatgaacagcctgagagccgaagacacggccgtatattactgtgcgaaaccgtttccgtattttgactactggggccagggaaccctggtcaccgtctcgagt

SEQ ID NO: 3 - protein, 5 aa, Artificial Sequence
  Synthetic peptide sequence
SFSMS

SEQ ID NO: 4 - protein, 7 aa, Artificial Sequence
  Synthetic peptide sequence
GFTFSSF

SEQ ID NO: 5 - protein, 17 aa, Artificial Sequence
  Synthetic peptide sequence
SISGSSGTTYYADSVKG

SEQ ID NO: 6 - protein, 6 aa, Artificial Sequence
  Synthetic peptide sequence
SGSSGT

SEQ ID NO: 7 - protein, 7 aa, Artificial Sequence
  Synthetic peptide sequence
PFPYFDY

SEQ ID NO: 8 - protein, 446 aa, Artificial Sequence
  Synthetic peptide sequence
EVQLLESGGGLVQPGGSLRLSCAASGFTFSSFSMSWVRQAPGKGLEWVSSISGSSGTTYYADSVKGRFTISRDNSKNTLYLQMNSLRAEDTAVYYCAKPFPYFDYWGQGTLVTVSSASTKGPSVFPLAPSSKSTSGGTAALGCLVKDYFPEPVTVSWNSGALTSGVHTFPAVLQSSGLYSLSSVVTVPSSSLGTQTYICNVNHKPSNTKVDKKVEPKSCDKTHTCPPCPAPELLGGPSVFLFPPKPKDTLMISRTPEVTCVVVDVSHEDPEVKFNWYVDGVEVHNAKTKPREEQYNSTYRVVSVLTVLHQDWLNGKEYKCKVSNKALPAPIEKTISKAKGQPREPQVYTLPPSRDELTKNQVSLTCLVKGFYPSDIAVEWESNGQPENNYKTTPPVLDSDGSFFLYSKLTVDKSRWQQGNVFSCSVMHEALHNHYTQKSLSLSPGK

SEQ ID NO: 9 - DNA, 1338 bp, Artificial Sequence
  Synthetic nucleotide sequence
gaggtgcagctgttggagtctgggggaggcttggtacagcctggggggtccctgagactctcctgtgcagcctctggattcacctttagcagtttttcgatgagctgggtccgccaggctccagggaaggggctggagtgggtctcatctattagtggtagttcgggtaccacatactacgcagactccgtgaagggccggttcaccatctccagagacaattccaagaacacgctgtatctgcaaatgaacagcctgagagccgaagacacggccgtatattactgtgcgaaaccgtttccgtattttgactactggggccagggaaccctggtcaccgtctcgagtgcgtcgaccaagggcccatcggtcttccccctggcaccctcctccaagagcacctctgggggcacagcggccctgggctgcctggtcaaggactacttccccgaaccggtgacggtgtcgtggaactcaggcgccctgaccagcggcgtgcacaccttcccggctgtcctacagtcctcaggactctactccctcagcagcgtggtgaccgtgccctccagcagcttgggcacccagacctacatctgcaacgtgaatcacaagcccagcaacaccaaggtggacaagaaagttgagcccaaatcttgtgacaaaactcacacatgcccaccgtgcccagcacctgaactcctggggggaccgtcagtcttcctcttccccccaaaacccaaggacaccctcatgatctcccggacccctgaggtcacatgcgtggtggtggacgtgagccacgaagaccctgaggtcaagttcaactggtacgtggacggcgtggaggtgcataatgccaagacaaagccgcgggaggagcagtacaacagcacgtaccgtgtggtcagcgtcctcaccgtcctgcaccaggactggctgaatggcaaggagtacaagtgcaaggtctccaacaaagccctcccagcccccatcgagaaaaccatctccaaagccaaagggcagccccgagaaccacaggtgtacaccctgcccccatcccgggatgagctgaccaagaaccaggtcagcctgacctgcctggtcaaaggcttctatcccagcgacatcgccgtggagtgggagagcaatgggcagccggagaacaactacaagaccacgcctcccgtgctggactccgacggctccttcttcctctacagcaagctcaccgtggacaagagcaggtggcagcaggggaacgtcttctcatgctccgtgatgcatgaggctctgcacaaccactacacgcagaagagcctctccctgtctccgggtaaa

SEQ ID NO: 10 - protein, 108 aa, Artificial Sequence [sequence omitted]

SEQ ID NO: 11 - DNA, 324 bp, Artificial Sequence
  Synthetic nucleotide sequence
gaaattgtgttaacgcagtctccaggcaccctgtctttgtctccaggggaaagagccaccctctcctgcagggccagtcagagtgttagcagcagctttttagcctggtaccagcagaaacctggccaggctcccaggctcctcatctattatgcatccagcagggccactggcatcccagacaggttcagtggcagtgggtctgggacagacttcactctcaccatcagcagactggagcctgaagattttgcagtgtattactgtcagcagacgggtcgtattccgccgacgttcggccaagggaccaaggtggaaatcaaa

SEQ ID NO: 12 - protein, 12 aa, Artificial Sequence
  Synthetic peptide sequence
RASQSVSSSFLA

SEQ ID NO: 13 - protein, 7 aa, Artificial Sequence
  Synthetic peptide sequence
YASSRAT

SEQ ID NO: 14 - protein, 9 aa, Artificial Sequence
  Synthetic peptide sequence
QQTGRIPPT

SEQ ID NO: 15 - protein, 215 aa, Artificial Sequence
  Synthetic peptide sequence
EIVLTQSPGTLSLSPGERATLSCRASQSVSSSFLAWYQQKPGQAPRLLIYYASSRATGIPDRFSGSGSGTDFTLTISRLEPEDFAVYYCQQTGRIPPTFGQGTKVEIKRTVAAPSVFIFPPSDEQLKSGTASVVCLLNNFYPREAKVQWKVDNALQSGNSQESVTEQDSKDSTYSLSSTLTLSKADYEKHKVYACEVTHQGLSSPVTKSFNRGEC

SEQ ID NO: 16 - DNA, 645 bp, Artificial Sequence
  Synthetic nucleotide sequence
gaaattgtgttaacgcagtctccaggcaccctgtctttgtctccaggggaaagagccaccctctcctgcagggccagtcagagtgttagcagcagctttttagcctggtaccagcagaaacctggccaggctcccaggctcctcatctattatgcatccagcagggccactggcatcccagacaggttcagtggcagtgggtctgggacagacttcactctcaccatcagcagactggagcctgaagattttgcagtgtattactgtcagcagacgggtcgtattccgccgacgttcggccaagggaccaaggtggaaatcaaacgtacggtggctgcaccatctgtcttcatcttcccgccatctgatgagcagttgaaatctggaactgcctctgttgtgtgcctgctgaataacttctatcccagagaggccaaagtacagtggaaggtggataacgccctccaatcgggtaactcccaggagagtgtcacagagcaggacagcaaggacagcacctacagcctcagcagcaccctgacgctgagcaaagcagactacgagaaacacaaagtctacgcctgcgaagtcacccatcagggcctgagctcgcccgtcacaaagagcttcaacaggggagagtgt

SEQ ID NO: 17 - protein, 445 aa, Artificial Sequence
  Synthetic peptide sequence
EVQLLESGGGLVQPGGSLRLSCAASGFTFSSFSMSWVRQAPGKGLEWVSSISGSSGTTYYADSVKGRFTISRDNSKNTLYLQMNSLRAEDTAVYYCAKPFPYFDYWGQGTLVTVSSASTKGPSVFPLAPSSKSTSGGTAALGCLVKDYFPEPVTVSWNSGALTSGVHTFPAVLQSSGLYSLSSVVTVPSSSLGTQTYICNVNHKPSNTKVDKKVEPKSCDKTHTCPPCPAPELLGGPSVFLFPPKPKDTLMISRTPEVTCVVVDVSHEDPEVKFNWYVDGVEVHNAKTKPREEQYNSTYRVVSVLTVLHQDWLNGKEYKCKVSNKALPAPIEKTISKAKGQPREPQVYTLPPSREEMTKNQVSLTCLVKGFYPSDIAVEWESNGQPENNYKTTPPVLDSDGSFFLYSKLTVDKSRWQQGNVFSCSVMHEALHNHYTQKSLSLSPG

SEQ ID NO: 18 - DNA, 1335 bp, Artificial Sequence
  Synthetic nucleotide sequence
gaggtgcagctgttggagtctgggggaggcttggtacagcctggggggtccctgagactctcctgtgcagcctctggattcacctttagcagtttttcgatgagctgggtccgccaggctccagggaaggggctggagtgggtctcatctattagtggtagttcgggtaccacatactacgcagactccgtgaagggccggttcaccatctccagagacaattccaagaacacgctgtatctgcaaatgaacagcctgagagccgaagacacggccgtatattactgtgcgaaaccgtttccgtattttgactactggggccagggaaccctggtcaccgtctcgagtgcgtcgaccaagggcccatcggtcttccccctggcaccctcctccaagagcacctctgggggcacagcggccctgggctgcctggtcaaggactacttccccgaaccggtgacggtgtcgtggaactcaggcgccctgaccagcggcgtgcacaccttcccggctgtcctacagtcctcaggactctactccctcagcagcgtggtgaccgtgccctccagcagcttgggcacccagacctacatctgcaacgtgaatcacaagcccagcaacaccaaggtggacaagaaagttgagcccaaatcttgtgacaaaactcacacatgcccaccgtgcccagcacctgaactcctggggggaccgtcagtcttcctcttccccccaaaacccaaggacaccctcatgatctcccggacccctgaggtcacatgcgtggtggtggacgtgagccacgaagaccctgaggtcaagttcaactggtacgtggacggcgtggaggtgcataatgccaagacaaagccgcgggaggagcagtacaacagcacgtaccgtgtggtcagcgtcctcaccgtcctgcaccaggactggctgaatggcaaggagtacaagtgcaaggtctccaacaaagccctcccagcccccatcgagaaaaccatctccaaagccaaagggcagccccgagaaccacaggtgtacaccctgcccccatcccgggaggagatgaccaagaaccaggtcagcctgacctgcctggtcaaaggcttctatcccagcgacatcgccgtggagtgggagagcaatgggcagccggagaacaactacaagaccacgcctcccgtgctggactccgacggctccttcttcctctatagcaagctcaccgtggacaagagcaggtggcagcaggggaacgtcttctcatgctccgtgatgcatgaggctctgcacaaccactacacgcagaagagcctctccctgtccccgggt

SEQ ID NO: 19 - protein, 445 aa, Artificial Sequence
  Synthetic peptide sequence
EVQLLESGGGLVQPGGSLRLSCAASGFTFSSFSMSWVRQAPGKGLEWVSSISGSSGTTYYADSVKGRFTISRDNSKNTLYLQMNSLRAEDTAVYYCAKPFPYFDYWGQGTLVTVSSASTKGPSVFPLAPSSKSTSGGTAALGCLVKDYFPEPVTVSWNSGALTSGVHTFPAVLQSSGLYSLSSVVTVPSSSLGTQTYICNVNHKPSNTKVDKKVEPKSCDKTHTCPPCPAPELLGGPSVFLFPPKPKDTLMISRTPEVTCVVVDVSHEDPEVKFNWYVDGVEVHNAKTCPREEQYNSTYRVVSVLTVLHQDWLNGKEYKCKVSNKALPAPIEKTISKAKGQPREPQVYTLPPSREEMTKNQVSLTCLVKGFYPSDIAVEWESNGQPENNYKTTPPVLDSDGSFFLYSKLTVDKSRWQQGNVFSCSVMHEALHNHYTQKSLSLSPG

SEQ ID NO: 20 - DNA, 1335 bp, Artificial Sequence
  Synthetic nucleotide sequence
gaggtgcagctgttggagtctgggggaggcttggtacagcctggggggtccctgagactctcctgtgcagcctctggattcacctttagcagtttttcgatgagctgggtccgccaggctccagggaaggggctggagtgggtctcatctattagtggtagttcgggtaccacatactacgcagactccgtgaagggccggttcaccatctccagagacaattccaagaacacgctgtatctgcaaatgaacagcctgagagccgaagacacggccgtatattactgtgcgaaaccgtttccgtattttgactactggggccagggaaccctggtcaccgtctcgagtgcgtcgaccaagggcccatcggtcttccccctggcaccctcctccaagagcacctctgggggcacagcggccctgggctgcctggtcaaggactacttccccgaaccggtgacggtgtcgtggaactcaggcgccctgaccagcggcgtgcacaccttcccggctgtcctacagtcctcaggactctactccctcagcagcgtggtgaccgtgccctccagcagcttgggcacccagacctacatctgcaacgtgaatcacaagcccagcaacaccaaggtggacaagaaagttgagcccaaatcttgtgacaaaactcacacatgcccaccgtgcccagcacctgaactcctggggggaccgtcagtcttcctcttccccccaaaacccaaggacaccctcatgatctcccggacccctgaggtcacatgcgtggtggtggacgtgagccacgaagaccctgaggtcaagttcaactggtacgtggacggcgtggaggtgcataatgccaagacatgcccgcgggaggagcagtacaacagcacgtaccgtgtggtcagcgtcctcaccgtcctgcaccaggactggctgaatggcaaggagtacaagtgcaaggtctccaacaaagccctcccagcccccatcgagaaaaccatctccaaagccaaagggcagccccgagaaccacaggtgtacaccctgcccccatcccgggaggagatgaccaagaaccaggtcagcctgacctgcctggtcaaaggcttctatcccagcgacatcgccgtggagtgggagagcaatgggcagccggagaacaactacaagaccacgcctcccgtgctggactccgacggctccttcttcctctatagcaagctcaccgtggacaagagcaggtggcagcaggggaacgtcttctcatgctccgtgatgcatgaggctctgcacaaccactacacgcagaagagcctctccctgtccccgggt

SEQ ID NO: 21 - protein, 116 aa, Artificial Sequence
  Synthetic peptide sequence
EVQLLESGGGLVQPGGSLRLSCAASGFTFSSFSMSWVRQAPGKGLEWVSSISGSSGTTYYADSVKGRFTISRDNSKNTLYLQMNSLRAEDTAVYYCARPFPYFDYWGQGTLVTVSS

SEQ ID NO: 22 - DNA, 348 bp, Artificial Sequence
  Synthetic nucleotide sequence
gaggtgcagctgttggagtctgggggaggcttggtacagcctggggggtccctgagactctcctgtgcagcctctggattcacctttagcagtttttcgatgagctgggtccgccaggctccagggaaggggctggagtgggtctcatctattagtggtagttcgggtaccacatactacgcagactccgtgaagggccggttcaccatctccagagacaattccaagaacacgctgtatctgcaaatgaacagcctgagagccgaagacacggccgtatattactgtgcgagaccgtttccgtattttgactactggggccagggaaccctggtcaccgtctcgagt

SEQ ID NO: 23 - protein, 445 aa, Artificial Sequence
  Synthetic peptide sequence
EVQLLESGGGLVQPGGSLRLSCAASGFTFSSFSMSWVRQAPGKGLEWVSSISGSSGTTYYADSVKGRFTISRDNSKNTLYLQMNSLRAEDTAVYYCARPFPYFDYWGQGTLVTVSSASTKGPSVFPLAPSSKSTSGGTAALGCLVKDYFPEPVTVSWNSGALTSGVHTFPAVLQSSGLYSLSSVVTVPSSSLGTQTYICNVNHKPSNTKVDKKVEPKSCDKTHTCPPCPAPELLGGPSVFLFPPKPKDTLMISRTPEVTCVVVDVSHEDPEVKFNWYVDGVEVHNAKTKPREEQYNSTYRVVSVLTVLHQDWLNGKEYKCKVSNKALPAPIEKTISKAKGQPREPQVYTLPPSREEMTKNQVSLTCLVKGFYPSDIAVEWESNGQPENNYKTTPPVLDSDGSFFLYSKLTVDKSRWQQGNVFSCSVMHEALHNHYTQKSLSLSPG

SEQ ID NO: 24 - DNA, 1335 bp, Artificial Sequence
  Synthetic nucleotide sequence
gaggtgcagctgttggagtctgggggaggcttggtacagcctggggggtccctgagactctcctgtgcagcctctggattcacctttagcagtttttcgatgagctgggtccgccaggctccagggaaggggctggagtgggtctcatctattagtggtagttcgggtaccacatactacgcagactccgtgaagggccggttcaccatctccagagacaattccaagaacacgctgtatctgcaaatgaacagcctgagagccgaagacacggccgtatattactgtgcgagaccgtttccgtattttgactactggggccagggaaccctggtcaccgtctcgagtgcgtcgaccaagggcccatcggtcttccccctggcaccctcctccaagagcacctctgggggcacagcggccctgggctgcctggtcaaggactacttccccgaaccggtgacggtgtcgtggaactcaggcgccctgaccagcggcgtgcacaccttcccggctgtcctacagtcctcaggactctactccctcagcagcgtggtgaccgtgccctccagcagcttgggcacccagacctacatctgcaacgtgaatcacaagcccagcaacaccaaggtggacaagaaagttgagcccaaatcttgtgacaaaactcacacatgcccaccgtgcccagcacctgaactcctggggggaccgtcagtcttcctcttccccccaaaacccaaggacaccctcatgatctcccggacccctgaggtcacatgcgtggtggtggacgtgagccacgaagaccctgaggtcaagttcaactggtacgtggacggcgtggaggtgcataatgccaagacaaagccgcgggaggagcagtacaacagcacgtaccgtgtggtcagcgtcctcaccgtcctgcaccaggactggctgaatggcaaggagtacaagtgcaaggtctccaacaaagccctcccagcccccatcgagaaaaccatctccaaagccaaagggcagccccgagaaccacaggtgtacaccctgcccccatcccgggaggagatgaccaagaaccaggtcagcctgacctgcctggtcaaaggcttctatcccagcgacatcgccgtggagtgggagagcaatgggcagccggagaacaactacaagaccacgcctcccgtgctggactccgacggctccttcttcctctatagcaagctcaccgtggacaagagcaggtggcagcaggggaacgtcttctcatgctccgtgatgcatgaggctctgcacaaccactacacgcagaagagcctctccctgtccccgggt

SEQ ID NO: 25 - protein, 445 aa, Artificial Sequence
  Synthetic peptide sequence
EVQLLESGGGLVQPGGSLRLSCAASGFTFSSFSMSWVRQAPGKGLEWVSSISGSSGTTYYADSVKGRFTISRDNSKNTLYLQMNSLRAEDTAVYYCARPFPYFDYWGQGTLVTVSSASTKGPSVFPLAPSSKSTSGGTAALGCLVKDYFPEPVTVSWNSGALTSGVHTFPAVLQSSGLYSLSSVVTVPSSSLGTQTYICNVNHKPSNTKVDKKVEPKSCDKTHTCPPCPAPELLGGPSVFLFPPKPKDTLMISRTPEVTCVVVDVSHEDPEVKFNWYVDGVEVHNAKTCPREEQYNSTYRVVSVLTVLHQDWLNGKEYKCKVSNKALPAPIEKTISKAKGQPREPQVYTLPPSREEMTKNQVSLTCLVKGFYPSDIAVEWESNGQPENNYKTTPPVLDSDGSFFLYSKLTVDKSRWQQGNVFSCSVMHEALHNHYTQKSLSLSPG

SEQ ID NO: 26 - DNA, 1335 bp, Artificial Sequence
  Synthetic nucleotide sequence
gaggtgcagctgttggagtctgggggaggcttggtacagcctggggggtccctgagactctcctgtgcagcctctggattcacctttagcagtttttcgatgagctgggtccgccaggctccagggaaggggctggagtgggtctcatctattagtggtagttcgggtaccacatactacgcagactccgtgaagggccggttcaccatctccagagacaattccaagaacacgctgtatctgcaaatgaacagcctgagagccgaagacacggccgtatattactgtgcgagaccgtttccgtattttgactactggggccagggaaccctggtcaccgtctcgagtgcgtcgaccaagggcccatcggtcttccccctggcaccctcctccaagagcacctctgggggcacagcggccctgggctgcctggtcaaggactacttccccgaaccggtgacggtgtcgtggaactcaggcgccctgaccagcggcgtgcacaccttcccggctgtcctacagtcctcaggactctactccctcagcagcgtggtgaccgtgccctccagcagcttgggcacccagacctacatctgcaacgtgaatcacaagcccagcaacaccaaggtggacaagaaagttgagcccaaatcttgtgacaaaactcacacatgcccaccgtgcccagcacctgaactcctggggggaccgtcagtcttcctcttccccccaaaacccaaggacaccctcatgatctcccggacccctgaggtcacatgcgtggtggtggacgtgagccacgaagaccctgaggtcaagttcaactggtacgtggacggcgtggaggtgcataatgccaagacatgcccgcgggaggagcagtacaacagcacgtaccgtgtggtcagcgtcctcaccgtcctgcaccaggactggctgaatggcaaggagtacaagtgcaaggtctccaacaaagccctcccagcccccatcgagaaaaccatctccaaagccaaagggcagccccgagaaccacaggtgtacaccctgcccccatcccgggaggagatgaccaagaaccaggtcagcctgacctgcctggtcaaaggcttctatcccagcgacatcgccgtggagtgggagagcaatgggcagccggagaacaactacaagaccacgcctcccgtgctggactccgacggctccttcttcctctatagcaagctcaccgtggacaagagcaggtggcagcaggggaacgtcttctcatgctccgtgatgcatgaggctctgcacaaccactacacgcagaagagcctctccctgtcccccgga

SEQ ID NO: 27 - protein, 445 aa, Artificial Sequence
  Synthetic peptide sequence
EVQLLESGGGLVQPGGSLRLSCAASGFTFSSFSMSWVRQAPGKGLEWVSSISGSSGTTYYADSVKGRFTISRDNSKNTLYLQMNSLRAEDTAVYYCAKPFPYFDYWGQGTLVTVSSASTKGPSVFPLAPSSKSTSGGTAALGCLVKDYFPEPVTVSWNSGALTSGVHTFPAVLQSSGLYSLSSVVTVPSSSLGTQTYICNVNHKPSNTKVDKKVEPKSCDRTHTCPPCPAPELLGGPSVFLFPPKPKDTLMISRTPEVTCVVVDVSHEDPEVKFNWYVDGVEVHNAKTKPRELLQGSTYRVVSVLTVLHQDWLNGKEYKCKVSNKALPAPIEKTISKAKGQPREPQVYTLPPSREEMTKNQVSLTCLVKGFYPSDIAVEWESNGQPENNYKTTPPVLDSDGSFFLYSKLTVDKSRWQQGNVFSCSVMHEALHNHYTQKSLSLSPG

SEQ ID NO: 28 - DNA, 1335 bp, Artificial Sequence
  Synthetic nucleotide sequence
gaggtgcagctgttggagtctgggggaggcttggtacagcctggggggtccctgagactctcctgtgcagcctctggattcacctttagcagtttttcgatgagctgggtccgccaggctccagggaaggggctggagtgggtctcatctattagtggtagttcgggtaccacatactacgcagactccgtgaagggccggttcaccatctccagagacaattccaagaacacgctgtatctgcaaatgaacagcctgagagccgaagacacggccgtatattactgtgcgaaaccgtttccgtattttgactactggggccagggaaccctggtcaccgtctcgagtgcgtcgaccaagggcccatcggtcttccccctggcaccctcctccaagagcacctctgggggcacagcggccctgggctgcctggtcaaggactacttccccgaaccggtgacggtgtcgtggaactcaggcgccctgaccagcggcgtgcacaccttcccggctgtcctacagtcctcaggactctactccctcagcagcgtagtgaccgtgccctccagcagcttgggcacccagacctacatctgcaacgtgaatcacaagcccagcaacaccaaggtggacaagaaagttgagcccaaatcttgtgaccgcactcacacatgcccaccgtgcccagcacctgaactcctggggggaccgtcagtcttcctcttccccccaaaacccaaggacaccctcatgatctcccggacccctgaggtcacatgcgtggtggtggacgtgagccacgaagaccctgaggtcaagttcaactggtacgtggacggcgtggaggtgcataatgccaagacaaagccgcgggagctgctgcaggggagcacgtaccgtgtggtcagcgtcctcaccgtcctgcaccaggactggctgaatggcaaggagtacaagtgcaaggtctccaacaaagccctcccagcccccatcgagaaaaccatctccaaagccaaagggcagccccgagaaccacaggtgtacaccctgcccccatcccgggaggagatgaccaagaaccaggtcagcctgacctgcctggtcaaaggcttctatcccagcgacatcgccgtggagtgggagagcaatgggcagccggagaacaactacaagaccacgcctcccgtgctggactccgacggctccttcttcctctatagcaagctcaccgtggacaagagcaggtggcagcaggggaacgtcttctcatgctccgtgatgcatgaggctctgcacaaccactacacgcagaagagcctctccctgtctccgggt

SEQ ID NO: 29 - protein, 445 aa, Artificial Sequence
  Synthetic peptide sequence
EVQLLESGGGLVQPGGSLRLSCAASGFTFSSFSMSWVRQAPGKGLEWVSSISGSSGTTYYADSVKGRFTISRDNSKNTLYLQMNSLRAEDTAVYYCARPFPYFDYWGQGTLVTVSSASTKGPSVFPLAPSSKSTSGGTAALGCLVKDYFPEPVTVSWNSGALTSGVHTFPAVLQSSGLYSLSSVVTVPSSSLGTQTYICNVNHKPSNTKVDKKVEPKSCDRTHTCPPCPAPELLGGPSVFLFPPKPKDTLMISRTPEVTCVVVDVSHEDPEVKFNWYVDGVEVHNAKTKPRELLQGSTYRVVSVLTVLHQDWLNGKEYKCKVSNKALPAPIEKTISKAKGQPREPQVYTLPPSREEMTKNQVSLTCLVKGFYPSDIAVEWESNGQPENNYKTTPPVLDSDGSFFLYSKLTVDKSRWQQGNVFSCSVMHEALHNHYTQKSLSLSPG

SEQ ID NO: 30 - DNA, 1335 bp, Artificial Sequence
  Synthetic nucleotide sequence
gaggtgcagctgttggagtctgggggaggcttggtacagcctggggggtccctgagactctcctgtgcagcctctggattcacctttagcagtttttcgatgagctgggtccgccaggctccagggaaggggctggagtgggtctcatctattagtggtagttcgggtaccacatactacgcagactccgtgaagggccggttcaccatctccagagacaattccaagaacacgctgtatctgcaaatgaacagcctgagagccgaagacacggccgtatattactgtgcgagaccgtttccgtattttgactactggggccagggaaccctggtcaccgtctcgagtgcgtcgaccaagggcccatcggtcttccccctggcaccctcctccaagagcacctctgggggcacagcggccctgggctgcctggtcaaggactacttccccgaaccggtgacggtgtcgtggaactcaggcgccctgaccagcggcgtgcacaccttcccggctgtcctacagtcctcaggactctactccctcagcagcgtagtgaccgtgccctccagcagcttgggcacccagacctacatctgcaacgtgaatcacaagcccagcaacaccaaggtggacaagaaagttgagcccaaatcttgtgaccgcactcacacatgcccaccgtgcccagcacctgaactcctggggggaccgtcagtcttcctcttccccccaaaacccaaggacaccctcatgatctcccggacccctgaggtcacatgcgtggtggtggacgtgagccacgaagaccctgaggtcaagttcaactggtacgtggacggcgtggaggtgcataatgccaagacaaagccgcgggagctgctgcaggggagcacgtaccgtgtggtcagcgtcctcaccgtcctgcaccaggactggctgaatggcaaggagtacaagtgcaaggtctccaacaaagccctcccagcccccatcgagaaaaccatctccaaagccaaagggcagccccgagaaccacaggtgtacaccctgcccccatcccgggaggagatgaccaagaaccaggtcagcctgacctgcctggtcaaaggcttctatcccagcgacatcgccgtggagtgggagagcaatgggcagccggagaacaactacaagaccacgcctcccgtgctggactccgacggctccttcttcctctatagcaagctcaccgtggacaagagcaggtggcagcaggggaacgtcttctcatgctccgtgatgcatgaggctctgcacaaccactacacgcagaagagcctctccctgtcccccgga

SEQ ID NO: 31 - protein, 215 aa, Artificial Sequence
  Synthetic peptide sequence
EIVLTQSPGTLSLSPGERATLSCRASQSVSSSFLAWYQQKPGQAPRLLIYYASSRATGIPDRFSGSGSGTDFTLTISRLEPEDFAVYYCQQTGRIPPTFGQGTKVEIKRTVAAPSVFIFPPSDEQLKSGTASVVCLLNNFYPREAKVQWKVDNALQSGNSQESVTEQDSKDSTYSLSSTLTLSCADYEKHKVYACEVTHQGLSSPVTKSFNRGEC

SEQ ID NO: 32 - DNA, 645 bp, Artificial Sequence
  Synthetic nucleotide sequence
gaaattgtgttaacgcagtctccaggcaccctgtctttgtctccaggggaaagagccaccctctcctgcagggccagtcagagtgttagcagcagctttttagcctggtaccagcagaaacctggccaggctcccaggctcctcatctattatgcatccagcagggccactggcatcccagacaggttcagtggcagtgggtctgggacagacttcactctcaccatcagcagactggagcctgaagattttgcagtgtattactgtcagcagacgggtcgtattccgccgacgttcggccaagggaccaaggtggaaatcaaacgaactgtggctgcaccatctgtcttcatcttcccgccatctgatgagcagttgaaatctggaactgcctctgttgtgtgcctgctgaataacttctatcccagagaggccaaagtacagtggaaggtggataacgccctccaatcgggtaactcccaggagagtgtcacagagcaggacagcaaggacagcacctacagcctcagcagcaccctgacgctgagctgcgcagactacgagaaacacaaagtctacgcctgcgaagtcacccatcagggcctgagctcgcccgtcacaaagagcttcaacaggggagagtgt

SEQ ID NO: 33 - protein, 91 aa, Homo sapiens
EVPQLTDLSFVDITDSSIGLRWTPLNSSTIIGYRITVVAAGEGIPIFEDFVDSSVGYYTVTGLEPGIDYDISVITLINGGESAPTTLTQQT

SEQ ID NO: 34 - protein, 374 aa, Artificial Sequence
  Synthetic peptide sequence
VVTQLSPPTNLHLEANPDTGVLAVSWERSTTPDITGYRITTTPTNGQQGNSLEEVVHADQSSCTFDNLSPGLEYNVSVYTVKDDKESVPISDTIIPEVPQLTDLSFVDITDSSIGLRWTPLNSSTIIGYRITVVAAGEGIPIFEDFVDSSVGYYTVTGLEPGIDYDISVITLINGGESAPTTLTQQTAVPPPTDLRFTNIGPDTMRVTWAPPPSIDLTNFLVRYSPVKNEEDVAELSISPSDNAVVLTNLLPGTEYVVSVSSVYEQHESTPLRGRQKTGLDSPTGIDFSDITANSFTVHWIAPRATITGYRIRHHPEHFSGRPREDRVPHSRNSITLTNLTPGTEYVVSIVALNGREESPLLIGRSRSHHHHHH

SEQ ID NO: 35 - protein, 374 aa, Artificial Sequence
  Synthetic peptide sequence
VVTPLSPPTNLHLETNPDTGVLTVSWERSTTPDITGYRITTTPTNGQQGYSLEEVVHADQSSCTFDNLSPGLEYNVSVYTVKDDKESVPISDTIIPEVPQLTDLSFVDITDSSIGLRWTPLNSSTIIGYRITVVAAGEGIPIFEDFVDSSVGYYTVTGLEPGIDYDISVITLINGGESAPTTLTQQTAVPPPTDLRFTNIGPDTMRVTWAPPPSIDLTNFLVRYSPVKNEEDVAELSISPSDNAVVLTNLLPGTEYVVSVSSVYEQHESTPLRGRQKTGLDSPTGIDFSDITANSFTVHWIAPRATITGYRIRHHPEHMSGRPREDRVPPSRNSITLTNLTPGTEYVVSIVALNGREESPLLIGRSRSHHHHHH

SEQ ID NO: 36 - protein, 374 aa, Artificial Sequence
  Synthetic peptide sequence
VVTPLSPPTNLHLEANPDTGVLTVSWERSTTPDITGYRITTTPTNGQQGTALEEVVHADQSSCTFENLNPGLEYNVSVYTVKDDKESAPISDTVIPEVPQLTDLSFVDITDSSIGLRWTPLNSSTIIGYRITVVAAGEGIPIFEDFVDSSVGYYTVTGLEPGIDYDISVITLINGGESAPTTLTQQTAVPPPTDLRFTNIGPDTMRVTWAPPPSIELTNLLVRYSPVKNEEDVAELSISPSDNAVVLTNLLPGTEYLVSVSSVYEQHESIPLRGRQKTGLDSPTGFDSSDVTANSFTVHWVAPRAPITGYIIRHHAEHSAGRPRQDRVPPSRNSITLTNLNPGTEYIVTIIAVNGREESPPLIGRSRSHHHHHH

SEQ ID NO: 37 - protein, 107 aa, Artificial Sequence [sequence omitted]

SEQ ID NO: 38 - protein, 106 aa, Artificial Sequence
  Synthetic peptide sequence
GQPKANPTVTLFPPSSEELQANKATLVCLISDFYPGAVTVAWKADGSPVKAGVETTKPSKQSNNKYAASSYLSLTPEQWKSHRSYSCQVTHEGSTVEKTVAPTECS

SEQ ID NO: 39 - protein, 5 aa, Artificial Sequence
  Synthetic peptide sequence
LLQGG

SEQ ID NO: 40 - protein, 4 aa, Artificial Sequence
  Synthetic peptide sequence
LLQG

SEQ ID NO: 41 - protein, 6 aa, Artificial Sequence
  Synthetic peptide sequence
LSLSQG

SEQ ID NO: 42 - protein, 8 aa, Artificial Sequence
  Synthetic peptide sequence
GGGLLQGG

SEQ ID NO: 43 - protein, 5 aa, Artificial Sequence
  Synthetic peptide sequence
GLLQG

SEQ ID NO: 44 - protein, 10 aa, Artificial Sequence
  Synthetic peptide sequence
GSPLAQSHGG

SEQ ID NO: 45 - protein, 7 aa, Artificial Sequence
  Synthetic peptide sequence
GLLQGGG

SEQ ID NO: 46 - protein, 6 aa, Artificial Sequence
  Synthetic peptide sequence
GLLQGG

SEQ ID NO: 47 - protein, 4 aa, Artificial Sequence
  Synthetic peptide sequence
GLLQ

SEQ ID NO: 48 - protein, 8 aa, Artificial Sequence
  Synthetic peptide sequence
LLQLLQGA

SEQ ID NO: 49 - protein, 5 aa, Artificial Sequence
  Synthetic peptide sequence
LLQGA

SEQ ID NO: 50 - protein, 7 aa, Artificial Sequence
  Synthetic peptide sequence
LLQYQGA

SEQ ID NO: 51 - protein, 6 aa, Artificial Sequence
  Synthetic peptide sequence
LLQGSG

SEQ ID NO: 52 - protein, 6 aa, Artificial Sequence
  Synthetic peptide sequence
LLQYQG

SEQ ID NO: 53 - protein, 7 aa, Artificial Sequence
  Synthetic peptide sequence
LLQLLQG

SEQ ID NO: 54 - protein, 5 aa, Artificial Sequence
  Synthetic peptide sequence
SLLQG

SEQ ID NO: 55 - protein, 5 aa, Artificial Sequence
  Synthetic peptide sequence
LLQLQ

SEQ ID NO: 56 - protein, 6 aa, Artificial Sequence
  Synthetic peptide sequence
LLQLLQ

SEQ ID NO: 57 - protein, 5 aa, Artificial Sequence
  Synthetic peptide sequence
LLQGR